European Patent Application EP 4 339 206 A1, published March 20, 2024. Title: 抗抑制素抗体及其应用. Applicant: 宁波三生生物科技股份有限公司. The sequence listing filed with the application follows.

SEQUENCE LISTING (24 sequences)

SEQ ID NO: 1 - protein, 10 aa, synthetic construct
GFSLTTCGVN

SEQ ID NO: 2 - protein, 16 aa, synthetic construct
VIWRGGSTDYNAAFMS

SEQ ID NO: 3 - protein, 10 aa, synthetic construct
RKILLNGTVP

SEQ ID NO: 4 - protein, 11 aa, synthetic construct
RASQDISNYLN

SEQ ID NO: 5 - protein, 7 aa, synthetic construct
YTSRFHS

SEQ ID NO: 6 - protein, 9 aa, synthetic construct
QQGYSLPPT

SEQ ID NO: 7 - protein, 118 aa, synthetic construct
QVQLKQSGPSLVQPSQSLSITCTVSGFSLTTCGVNWVRQSPGKGLEWLGVIWRGGSTDYNAAFMSRMSITKDNSKSQVFFKMNSLPADDTAKYYFAKRKILLNGTVPTGQGTTLTVSS

SEQ ID NO: 8 - DNA, 354 bp, synthetic construct
  source 1..354: mol_type = other DNA
caggtgcagctgaagcagtccggaccctccctggtgcagccctcccagtccctgtccatcacctgcaccgtgtccggattctccctgaccacctgcggagtgaactgggtgagacagtcccccggaaagggactggagtggctgggagtgatctggagaggaggatccaccgactacaacgccgccttcatgtccagaatgtccatcaccaaggacaactccaagtcccaggtgttcttcaagatgaactccctgcccgccgacgacaccgccaagtactacttcgccaagagaaagatcctgctgaacggaaccgtgcccaccggacagggaaccaccctgaccgtgtcctcc

SEQ ID NO: 9 - protein, 107 aa, synthetic construct
DIQMTQTTSSLSASLGDRVTISCRASQDISNYLNWYQQKPDGTVKLLIYYTSRFHSGVPSRFSGSGSGTDYSLTISNLEQEDIATYFCQQGYSLPPTFGGGTKLEIK

SEQ ID NO: 10 - DNA, 321 bp, synthetic construct
  source 1..321: mol_type = other DNA
gacatccagatgacccagaccacctcctccctgtccgcctccctgggagacagagtgaccatctcctgcagagcctcccaggacatctccaactacctgaactggtaccagcagaagcccgacggaaccgtgaagctgctgatctactacacctccagattccactccggagtgccctccagattctccggatccggatccggaaccgactactccctgaccatctccaacctggagcaggaggacatcgccacctacttctgccagcagggatactccctgccccccaccttcggaggaggaaccaagctggagatcaag

SEQ ID NO: 11 - protein, 10 aa, synthetic construct
GYTFTDYSMH

SEQ ID NO: 12 - protein, 17 aa, synthetic construct
WINTETGEPTYADDFKG

SEQ ID NO: 13 - protein, 10 aa, synthetic construct
YGPPTYSLDY

SEQ ID NO: 14 - protein, 11 aa, synthetic construct
RASQGISNYLN

SEQ ID NO: 15 - protein, 7 aa, synthetic construct
YTSRLLS

SEQ ID NO: 16 - protein, 9 aa, synthetic construct
QQGYTLPFT

SEQ ID NO: 17 - protein, 119 aa, synthetic construct
EVKLVESGPELKKPGETVKISCKASGYTFTDYSMHWVKQAPGKGLKWMGWINTETGEPTYADDFKGRFAFSLETSASTAYLQINNLKNEDTATYFCAYYGPPTYSLDYWGQGASVTVSS

SEQ ID NO: 18 - DNA, 357 bp, synthetic construct
  source 1..357: mol_type = other DNA
gaggtgaagctggtggagtccggacccgagctgaagaagcccggagagaccgtgaagatctcctgcaaggcctccggatacaccttcaccgactactccatgcactgggtgaagcaggcccccggaaagggactgaagtggatgggatggatcaacaccgagaccggagagcccacctacgccgacgacttcaagggaagattcgccttctccctggagacctccgcctccaccgcctacctgcagatcaacaacctgaagaacgaggacaccgccacctacttctgcgcctactacggaccccccacctactccctggactactggggacagggagcctccgtgaccgtgtcctcc

SEQ ID NO: 19 - protein, 107 aa, synthetic construct
DIQMTQTTSSLSASLGDRVTISCRASQGISNYLNWYQQKPDGTVKLLIYYTSRLLSGVPSRFSGSGSGTDYSLTISNLEQEDIATYFCQQGYTLPFTFGSGTKLEIK

SEQ ID NO: 20 - DNA, 321 bp, synthetic construct
  source 1..321: mol_type = other DNA
gacatccagatgacccagaccacctcctccctgtccgcctccctgggagacagagtgaccatctcctgcagagcctcccagggaatctccaactacctgaactggtaccagcagaagcccgacggaaccgtgaagctgctgatctactacacctccagactgctgtccggagtgccctccagattctccggatccggatccggaaccgactactccctgaccatctccaacctggagcaggaggacatcgccacctacttctgccagcagggatacaccctgcccttcaccttcggatccggaaccaagctggagatcaag

SEQ ID NO: 21 - protein, 19 aa, synthetic construct
MEFGLSWVFLVALFRGVQC

SEQ ID NO: 22 - protein, 324 aa, synthetic construct
AKTTPPSVYPLAPGSAAQTNSMVTLGCLVKGYFPEPVTVTWNSGSLSSGVHTFPAVLQSDLYTLSSSVTVPSSPRPSETVTCNVAHPASSTKVDKKIVPRDCGCKPCICTVPEVSSVFIFPPKPKDVLTITLTPKVTCVVVDISKDDPEVQFSWFVDDVEVHTAQTQPREEQFNSTFRSVSELPIMHQDWLNGKEFKCRVNSAAFPAPIEKTISKTKGRPKAPQVYTIPPPKEQMAKDKVSLTCMITDFFPEDITVEWQWNGQPAENYKNTQPIMNTNGSYFVYSKLNVQKSNWEAGNTFTCSVLHEGLHNHHTEKSLSHSPGK

SEQ ID NO: 23 - protein, 107 aa, synthetic construct
RADAAPTVSIFPPSSEQLTSGGASVVCFLNNFYPKDINVKWKIDGSERQNGVLNSWTDQDSKDSTYSMSSTLTLTKDEYERHNSYTCEATHKTSTSPIVKSFNRNEC

SEQ ID NO: 24 - protein, 20 aa, synthetic construct
WPWSPAALRLLQRPPEEPAV